European Patent Application EP 4 400 117 A1, published July 17, 2024. Title: Screening method for Senolytic Agents. Applicant: 国立大学法人京都大学. The sequence listing filed with the application follows.

SEQUENCE LISTING (81 sequences)

SEQ ID NO: 1 - protein, 254 aa, Homo sapiens
MAAYKLVLIRHGESAWNLENRFSGWYDADLSPAGHEEAKRGGQALRDAGYEFDICFTSVQKRAIRTLWTVLDAIDQMWLPVVRTWRLNERHYGGLTGLNKAETAAKHGEAQVKIWRRSYDVPPPPMEPDHPFYSNISKDRRYADLTEDQLPSCESLKDTIARALPFWNEEIVPQIKEGKRVLIAAHGNSLRGIVKHLEGLSEEAIMELNLPTGIPIVYELDKNLKPIKPMQFLGDEETVRKAMEAVAAQGKAKK

SEQ ID NO: 2 - protein, 253 aa, Homo sapiens
MATHRLVMVRHGESTWNQENRFCGWFDAELSEKGTEEAKRGAKAIKDAKMEFDICYTSVLKRAIRTLWAILDGTDQMWLPVVRTWRLNERHYGGLTGLNKAETAAKHGEEQVKIWRRSFDIPPPPMDEKHPYYNSISKERRYAGLKPGELPTCESLKDTIARALPFWNEEIVPQIKAGKRVLIAAHGNSLRGIVKHLEGMSDQAIMELNLPTGIPIVYELNKELKPTKPMQFLGDEETVRKAMEAVAAQGKAK

SEQ ID NO: 3 - DNA, 765 bp, Homo sapiens
  source 1..765: mol_type = other DNA
atggccgcctacaaactggtgctgatccggcacggcgagagcgcatggaacctggagaaccgcttcagcggctggtacgacgccgacctgagcccggcgggccacgaggaggcgaagcgcggcgggcaggcgctacgagatgctggctatgagtttgacatctgcttcacctcagtgcagaagagagcgatccggaccctctggacagtgctagatgccattgatcagatgtggctgccagtggtgaggacttggcgcctcaatgagcggcactatgggggtctaaccggtctcaataaagcagaaactgctgcaaagcatggtgaggcccaggtgaagatctggaggcgctcctatgatgtcccaccacctccgatggagcccgaccatcctttctacagcaacatcagtaaggatcgcaggtatgcagacctcacagaagatcagctaccctcctgtgagagtctgaaggatactattgccagagctctgcccttctggaatgaagaaatagttccccagatcaaggaggggaaacgtgtactgattgcagcccatggcaacagcctccggggcattgtcaagcatctggagggtctctctgaagaggctatcatggagctgaacctgccgactggtattcccattgtctatgaattggacaagaacttgaagcctatcaagcccatgcagtttctgggggatgaagagacggtgcgcaaagccatggaagctgtggctgcccagggcaaggccaagaagtga

SEQ ID NO: 4 - DNA, 762 bp, Homo sapiens
  source 1..762: mol_type = other DNA
atggccactcaccgcctcgtgatggtccggcacggcgagagcacatggaaccaggagaaccgtttctgtggctggttcgatgcagagctgagtgaaaaggggaccgaggaggccaagcggggagccaaggccatcaaggatgccaagatggagtttgacatctgctacacgtcagtgctgaagcgggccatccgcaccctctgggccatcctggacggcacggaccagatgtggctgcctgtggtgcgcacttggcgcctcaatgagcggcattacgggggcctcacaggcctcaacaaggcagaaacggccgccaagcacggggaggagcaggtgaagatctggaggcgctccttcgacatcccgccgcccccgatggacgagaagcacccctactacaactccattagcaaggagcgtcggtacgcaggcctgaagcccggggaactccccacctgcgagagcctcaaggacaccattgcccgggccctgcccttctggaacgaggagattgttccccagatcaaggccggcaagcgagtgctcattgcagcccacgggaacagcctgcggggcattgtcaagcacctggaagggatgtcagaccaggcgatcatggagctgaacctgcccacggggatccccattgtgtatgagctgaacaaggagctgaagcccaccaagcccatgcagttcctgggtgatgaggaaacggtgcggaaggccatggaggctgtggctgcccagggcaaggccaagtga

SEQ ID NO: 5 - protein, 476 aa, Homo sapiens
MAVPFVEDWDLVQTLGEGAYGEVQLAVNRVTEEAVAVKIVDMKRAVDCPENIKKEICINKMLNHENVVKFYGHRREGNIQYLFLEYCSGGELFDRIEPDIGMPEPDAQRFFHQLMAGVVYLHGIGITHRDIKPENLLLDERDNLKISDFGLATVFRYNNRERLLNKMCGTLPYVAPELLKRREFHAEPVDVWSCGIVLTAMLAGELPWDQPSDSCQEYSDWKEKKTYLNPWKKIDSAPLALLHKILVENPSARITIPDIKKDRWYNKPLKKGAKRPRVTSGGVSESPSGFSKHIQSNLDFSPVNSASSEENVKYSSSQPEPRTGLSLWDTSPSYIDKLVQGISFSQPTCPDHMLLNSQLLGTPGSSQNPWQRLVKRMTRFFTKLDADKSYQCLKETCEKLGYQWKKSCMNQVTISTTDRRNNKLIFKVNLLEMDDKILVDFRLSKGDGLEFKRHFLKIKGKLIDIVSSQKIWLPAT

SEQ ID NO: 6 - DNA, 1431 bp, Homo sapiens
  source 1..1431: mol_type = other DNA
atggcagtgccctttgtggaagactgggacttggtgcaaaccctgggagaaggtgcctatggagaagttcaacttgctgtgaatagagtaactgaagaagcagtcgcagtgaagattgtagatatgaagcgtgccgtagactgtccagaaaatattaagaaagagatctgtatcaataaaatgctaaatcatgaaaatgtagtaaaattctatggtcacaggagagaaggcaatatccaatatttatttctggagtactgtagtggaggagagctttttgacagaatagagccagacataggcatgcctgaaccagatgctcagagattcttccatcaactcatggcaggggtggtttatctgcatggtattggaataactcacagggatattaaaccagaaaatcttctgttggatgaaagggataacctcaaaatctcagactttggcttggcaacagtatttcggtataataatcgtgagcgtttgttgaacaagatgtgtggtactttaccatatgttgctccagaacttctgaagagaagagaatttcatgcagaaccagttgatgtttggtcctgtggaatagtacttactgcaatgctcgctggagaattgccatgggaccaacccagtgacagctgtcaggagtattctgactggaaagaaaaaaaaacatacctcaacccttggaaaaaaatcgattctgctcctctagctctgctgcataaaatcttagttgagaatccatcagcaagaattaccattccagacatcaaaaaagatagatggtacaacaaacccctcaagaaaggggcaaaaaggccccgagtcacttcaggtggtgtgtcagagtctcccagtggattttctaagcacattcaatccaatttggacttctctccagtaaacagtgcttctagtgaagaaaatgtgaagtactccagttctcagccagaaccccgcacaggtctttccttatgggataccagcccctcatacattgataaattggtacaagggatcagcttttcccagcccacatgtcctgatcatatgcttttgaatagtcagttacttggcaccccaggatcctcacagaacccctggcagcggttggtcaaaagaatgacacgattctttaccaaattggatgcagacaaatcttatcaatgcctgaaagagacttgtgagaagttgggctatcaatggaagaaaagttgtatgaatcaggttactatatcaacaactgataggagaaacaataaactcattttcaaagtgaatttgttagaaatggatgataaaatattggttgacttccggctttctaagggtgatggattggagttcaagagacacttcctgaagattaaagggaagctgattgatattgtgagcagccagaagatttggcttcctgccacatga

SEQ ID NO: 7 - RNA, 19 nt, synthetic construct
  source 1..19: mol_type = other RNA
cactgattctgaaggcgaa

SEQ ID NO: 8 - RNA, 19 nt, synthetic construct
  source 1..19: mol_type = other RNA
acggctacgtggtaaagga

SEQ ID NO: 9 - RNA, 19 nt, synthetic construct
  source 1..19: mol_type = other RNA
cacctactgtgatgacaga

SEQ ID NO: 10 - RNA, 19 nt, synthetic construct
  source 1..19: mol_type = other RNA
caatagccctgaagactat

SEQ ID NO: 11 - DNA, 20 bp, synthetic construct
  source 1..20: mol_type = other DNA
ctggaccgtctcaaggtgtt

SEQ ID NO: 12 - DNA, 19 bp, synthetic construct
  source 1..19: mol_type = other DNA
gccccagataggcaaactt

SEQ ID NO: 13 - DNA, 21 bp, synthetic construct
  source 1..21: mol_type = other DNA
ggtgtcatcctcttccatgag

SEQ ID NO: 14 - DNA, 20 bp, synthetic construct
  source 1..20: mol_type = other DNA
gtagtctcgccatttgtccc

SEQ ID NO: 15 - DNA, 22 bp, synthetic construct
  source 1..22: mol_type = other DNA
ctttgtcaagctcatttcctgg

SEQ ID NO: 16 - DNA, 20 bp, synthetic construct
  source 1..20: mol_type = other DNA
tcttcctcttgtgctcttgc

SEQ ID NO: 17 - DNA, 22 bp, synthetic construct
  source 1..22: mol_type = other DNA
gcttctgggaacaaggttaaag

SEQ ID NO: 18 - DNA, 21 bp, synthetic construct
  source 1..21: mol_type = other DNA
ctgtggcagattgactcctac

SEQ ID NO: 19 - DNA, 20 bp, synthetic construct
  source 1..20: mol_type = other DNA
ggaggcgctcctatgatgtc

SEQ ID NO: 20 - DNA, 22 bp, synthetic construct
  source 1..22: mol_type = other DNA
atcttctgtgaggtctgcatac

SEQ ID NO: 21 - DNA, 20 bp, synthetic construct
  source 1..20: mol_type = other DNA
ttggagcagaggtttaccac

SEQ ID NO: 22 - DNA, 21 bp, synthetic construct
  source 1..21: mol_type = other DNA
ttcccaatagcagtcttcagc

SEQ ID NO: 23 - DNA, 20 bp, synthetic construct
  source 1..20: mol_type = other DNA
tgtggatgcagaagatggag

SEQ ID NO: 24 - DNA, 20 bp, synthetic construct
  source 1..20: mol_type = other DNA
gtgacttcccgacccagtag

SEQ ID NO: 25 - DNA, 21 bp, synthetic construct
  source 1..21: mol_type = other DNA
agttccagttcaacccaccaa

SEQ ID NO: 26 - DNA, 20 bp, synthetic construct
  source 1..20: mol_type = other DNA
ttgcagagcaaggcatcaga

SEQ ID NO: 27 - DNA, 20 bp, synthetic construct
  source 1..20: mol_type = other DNA
cgtggcctctaagatgaagg

SEQ ID NO: 28 - DNA, 20 bp, synthetic construct
  source 1..20: mol_type = other DNA
ccacttgagcttgttcacca

SEQ ID NO: 29 - DNA, 20 bp, synthetic construct
  source 1..20: mol_type = other DNA
ctgaccattccaccaaggtt

SEQ ID NO: 30 - DNA, 20 bp, synthetic construct
  source 1..20: mol_type = other DNA
agtcgaccacctcacctgtc

SEQ ID NO: 31 - DNA, 22 bp, synthetic construct
  source 1..22: mol_type = other DNA
gagaccttggtggaatacctgc

SEQ ID NO: 32 - DNA, 23 bp, synthetic construct
  source 1..23: mol_type = other DNA
acgaagatccaaaagccttgcac

SEQ ID NO: 33 - DNA, 22 bp, synthetic construct
  source 1..22: mol_type = other DNA
tcgaccgtcaacatgtgcagca

SEQ ID NO: 34 - DNA, 23 bp, synthetic construct
  source 1..23: mol_type = other DNA
ggctctgtgatggcaaactcatg

SEQ ID NO: 35 - DNA, 20 bp, synthetic construct
  source 1..20: mol_type = other DNA
ccactgagaacgagccagac

SEQ ID NO: 36 - DNA, 20 bp, synthetic construct
  source 1..20: mol_type = other DNA
gacagaaaggaaagcgcaac

SEQ ID NO: 37 - DNA, 20 bp, synthetic construct
  source 1..20: mol_type = other DNA
ctggtcatcctgggaacagt

SEQ ID NO: 38 - DNA, 20 bp, synthetic construct
  source 1..20: mol_type = other DNA
cttcttcatccgagcctgtc

SEQ ID NO: 39 - DNA, 20 bp, synthetic construct
  source 1..20: mol_type = other DNA
tccctgctgtctcgatcctc

SEQ ID NO: 40 - DNA, 20 bp, synthetic construct
  source 1..20: mol_type = other DNA
ggtcttcggctgcttggtaa

SEQ ID NO: 41 - DNA, 20 bp, synthetic construct
  source 1..20: mol_type = other DNA
gacgacctcaacgcacagta

SEQ ID NO: 42 - DNA, 22 bp, synthetic construct
  source 1..22: mol_type = other DNA
aggagtcccatgatgagattgt

SEQ ID NO: 43 - DNA, 21 bp, synthetic construct
  source 1..21: mol_type = other DNA
gttttccgcagctacgttttt

SEQ ID NO: 44 - DNA, 22 bp, synthetic construct
  source 1..22: mol_type = other DNA
gcagaggtaaggtgaccatctc

SEQ ID NO: 45 - DNA, 18 bp, synthetic construct
  source 1..18: mol_type = other DNA
gcacagcaacgcagatgc

SEQ ID NO: 46 - DNA, 19 bp, synthetic construct
  source 1..19: mol_type = other DNA
aagttccgatcccaccagg

SEQ ID NO: 47 - DNA, 24 bp, synthetic construct
  source 1..24: mol_type = other DNA
tctactttgccagcaaactggtgc

SEQ ID NO: 48 - DNA, 24 bp, synthetic construct
  source 1..24: mol_type = other DNA
tgtccagcccatgatggttctgat

SEQ ID NO: 49 - DNA, 20 bp, synthetic construct
  source 1..20: mol_type = other DNA
agaccctcctgtatgagcag

SEQ ID NO: 50 - DNA, 23 bp, synthetic construct
  source 1..23: mol_type = other DNA
gcattccaaagaatcgaagtcct

SEQ ID NO: 51 - DNA, 21 bp, synthetic construct
  source 1..21: mol_type = other DNA
gagccatctcagtgtgtggag

SEQ ID NO: 52 - DNA, 23 bp, synthetic construct
  source 1..23: mol_type = other DNA
gccagcattgccataaaagagtc

SEQ ID NO: 53 - DNA, 23 bp, synthetic construct
  source 1..23: mol_type = other DNA
tgctcggcaggcggaacttgtag

SEQ ID NO: 54 - DNA, 20 bp, synthetic construct
  source 1..20: mol_type = other DNA
ctttctccaaggacacaggg

SEQ ID NO: 55 - DNA, 20 bp, synthetic construct
  source 1..20: mol_type = other DNA
ctacgatgagctgcagactg

SEQ ID NO: 56 - DNA, 21 bp, synthetic construct
  source 1..21: mol_type = other DNA
gatgctacggtccatgctgtc

SEQ ID NO: 57 - DNA, 20 bp, synthetic construct
  source 1..20: mol_type = other DNA
cctgagcagaagagtttgga

SEQ ID NO: 58 - DNA, 20 bp, synthetic construct
  source 1..20: mol_type = other DNA
gctggaagtcgagtgtgcta

SEQ ID NO: 59 - DNA, 20 bp, synthetic construct
  source 1..20: mol_type = other DNA
agtcagttccttgtggagcc

SEQ ID NO: 60 - DNA, 19 bp, synthetic construct
  source 1..19: mol_type = other DNA
catgggttctgacggacat

SEQ ID NO: 61 - DNA, 20 bp, synthetic construct
  source 1..20: mol_type = other DNA
tgagagtagtgaggaacaag

SEQ ID NO: 62 - DNA, 19 bp, synthetic construct
  source 1..19: mol_type = other DNA
cgcagaatgagatgagttg

SEQ ID NO: 63 - DNA, 20 bp, synthetic construct
  source 1..20: mol_type = other DNA
ttgccttgaccctgaagctc

SEQ ID NO: 64 - DNA, 19 bp, synthetic construct
  source 1..19: mol_type = other DNA
tcagaagccagcgttcacc

SEQ ID NO: 65 - DNA, 20 bp, synthetic construct
  source 1..20: mol_type = other DNA
actacaagcagcactgccct

SEQ ID NO: 66 - DNA, 20 bp, synthetic construct
  source 1..20: mol_type = other DNA
agcagtcaaaggggatgaca

SEQ ID NO: 67 - DNA, 16 bp, synthetic construct
  source 1..16: mol_type = other DNA
cccaacgccccgaact

SEQ ID NO: 68 - DNA, 21 bp, synthetic construct
  source 1..21: mol_type = other DNA
gcagaagagctgctacgtgaa

SEQ ID NO: 69 - DNA, 22 bp, synthetic construct
  source 1..22: mol_type = other DNA
gataagctggagtcacagaagg

SEQ ID NO: 70 - DNA, 23 bp, synthetic construct
  source 1..23: mol_type = other DNA
ggaatgtccacaaactgatatgc

SEQ ID NO: 71 - DNA, 20 bp, synthetic construct
  source 1..20: mol_type = other DNA
ttgccttgaccctgaagctc

SEQ ID NO: 72 - DNA, 19 bp, synthetic construct
  source 1..19: mol_type = other DNA
tcagaagccagcgttcacc

SEQ ID NO: 73 - DNA, 21 bp, synthetic construct
  source 1..21: mol_type = other DNA
ccaaggtcaacctcctctctg

SEQ ID NO: 74 - DNA, 21 bp, synthetic construct
  source 1..21: mol_type = other DNA
ccaaagtagacctgcccagac

SEQ ID NO: 75 - DNA, 21 bp, synthetic construct
  source 1..21: mol_type = other DNA
gggtaccatgaagatctctgc

SEQ ID NO: 76 - DNA, 21 bp, synthetic construct
  source 1..21: mol_type = other DNA
tctagggagaggtaggcaaag

SEQ ID NO: 77 - protein, 30 aa, Homo sapiens
MTADKEKKRSSSERRKEKSRDAARCRRSKE

SEQ ID NO: 78 - protein, 30 aa, Mus musculus
MTADKEKKRSSSELRKEKSRDAARCRRSKE

SEQ ID NO: 79 - protein, 30 aa, Rattus norvegicus; identical to SEQ ID NO: 78

SEQ ID NO: 80 - protein, 30 aa, Gallus gallus; identical to SEQ ID NO: 77

SEQ ID NO: 81 - protein, 30 aa, Xenopus tropicalis
MTAEKEKKRNSSERRKEKSRDAARCRRSKE